European Patent Application EP 4 663 657 A1, published December 17, 2025. Title: IL-3 signaling inhibitor for use in a method of treatment of Long-COVID and/or Post-COVID syndrome. Applicant: Universitaet Regensburg. Application EP. The sequence listing filed with the application follows.

SEQUENCE LISTING (20 sequences)

SEQ ID NO: 1 - protein, 133 aa, synthetic construct
APMTQTTPLKTSWVNCSNMIDEIITHLKQPPLPLLDFNNLNGEDQDILMENNLRRPNLEAFNRAVKSLQNASAIESILKNLLPCLPLATAAPTRHPIHIKDGDWNEFRRKLTFYLKTLENAQAQQTTLSLAIF

SEQ ID NO: 2 - protein, 27 aa, synthetic construct
EIITHLKQPPLPLLDFNNLNGEDQDIL

SEQ ID NO: 3 - protein, 120 aa, synthetic construct
QVQLQQSGAEMVRPGVSVKIACKGSGFTFTDYALHWVKQSHAKSLEWIGLISTYYGDTTYNQRFKGKATMTVDKSSSTAYMELARLTSEDSAIYYCVITTVAGTDAMDYWGQGTSVTVSS

SEQ ID NO: 4 - protein, 5 aa, synthetic construct
DYALH

SEQ ID NO: 5 - protein, 17 aa, synthetic construct
LISTYYGDTTYNQRFKG

SEQ ID NO: 6 - protein, 11 aa, synthetic construct
TTVAGTDAMDY

SEQ ID NO: 7 - protein, 8 aa, synthetic construct
GFTFTDYA

SEQ ID NO: 8 - protein, 8 aa, synthetic construct
ISTYYGDT

SEQ ID NO: 9 - protein, 13 aa, synthetic construct
VITTVAGTDAMDY

SEQ ID NO: 10 - protein, 107 aa, synthetic construct
DIQMNQSPSSLSASLGDTITITCHASQNINVWLSWYQQKPGNIPKLLIYKASNLHTGVPSRFSGSGSGTGFTLTISSLQPEDIATYYCQQGYSYPYTFGGGTKLEIK

SEQ ID NO: 11 - protein, 11 aa, synthetic construct
HASQNINVWLS

SEQ ID NO: 12 - protein, 7 aa, synthetic construct
KASNLHT

SEQ ID NO: 13 - protein, 9 aa, synthetic construct
QQGYSYPYT

SEQ ID NO: 14 - protein, 6 aa, synthetic construct
QNINVW

SEQ ID NO: 15 - protein, 4 aa, synthetic construct
  MOTIF 1..3: note = LCDR2 (IMGT numbering) of P8C11 consists of the three amino acids: KAS. The N, also displayed in the sequence, is not a mandatory feature of the LCDR2.
KASN

SEQ ID NO: 16 - protein, 9 aa, synthetic construct
QQGYSYPYT

SEQ ID NO: 17 - protein, 120 aa, synthetic construct
QVQLVQSGAEVKKPGASVKVSCKGSGFTFTDYALHWVRQAPGQRLEWMGLISTYYGDTTYNQRFKGRVTMTVDKSTSTAYMELSSLRSEDTAVYYCVITTVAGTDAMDYWGQGTLVTVSS

SEQ ID NO: 18 - protein, 107 aa, synthetic construct
DIQMTQSPSSLSASVGDRVTITCHASQNINVWLSWYQQKPGKAPKLLIYKASNLHTGVPSRFSGSGSGTDFTFTISSLQPEDIATYYCQQGYSYPYTFGGGTKLEIK

SEQ ID NO: 19 - protein, 449 aa, synthetic construct
QVQLVQSGAEVKKPGASVKVSCKGSGFTFTDYALHWVRQAPGQRLEWMGLISTYYGDTTYNQRFKGRVTMTVDKSTSTAYMELSSLRSEDTAVYYCVITTVAGTDAMDYWGQGTLVTVSSASTKGPSVFPLAPSSKSTSGGTAALGCLVKDYFPEPVTVSWNSGALTSGVHTFPAVLQSSGLYSLSSVVTVPSSSLGTQTYICNVNHKPSNTKVDKRVEPKSCDKTHTCPPCPAPELLGGPSVFLFPPKPKDTLMISRTPEVTCVVVDVSHEDPEVKFNWYVDGVEVHNAKTKPREEQYNSTYRVVSVLTVLHQDWLNGKEYKCKVSNKALPAPIEKTISKAKGQPREPQVYTLPPSREEMTKNQVSLTCLVKGFYPSDIAVEWESNGQPENNYKTTPPVLDSDGSFFLYSKLTVDKSRWQQGNVFSCSVMHEALHNHYTQKSLSLSPG

SEQ ID NO: 20 - protein, 214 aa, synthetic construct
DIQMTQSPSSLSASVGDRVTITCHASQNINVWLSWYQQKPGKAPKLLIYKASNLHTGVPSRFSGSGSGTDFTFTISSLQPEDIATYYCQQGYSYPYTFGGGTKLEIKRTVAAPSVFIFPPSDEQLKSGTASVVCLLNNFYPREAKVQWKVDNALQSGNSQESVTEQDSKDSTYSLSSTLTLSKADYEKHKVYACEVTHQGLSSPVTKSFNRGEC